European Patent Application EP 4 778 582 A2, published July 22, 2026. Title: Treatment for SOD1 Associated Disease. Applicant: The Perron Institute for Neurological and Translational Science Limited. Application EP. The sequence listing filed with the application follows.

SEQUENCE LISTING (47 sequences)

SEQ ID NO: 1 - RNA, 25 nt, Homo sapiens
  source 1..25: mol_type = other RNA
gtccattactttcctttaagaaaag

SEQ ID NO: 2 - RNA, 25 nt, Homo sapiens
  source 1..25: mol_type = other RNA
gtcctttaatgcttccccacacctt

SEQ ID NO: 3 - RNA, 22 nt, Homo sapiens
  source 1..22: mol_type = other RNA
caggcttcagtcagtcctttaa

SEQ ID NO: 4 - RNA, 26 nt, Homo sapiens
  source 1..26: mol_type = other RNA
actcatgaacatggaatccatgcagg

SEQ ID NO: 5 - RNA, 21 nt, Homo sapiens
  source 1..21: mol_type = other RNA
acacccacctgctgtattatc

SEQ ID NO: 6 - RNA, 25 nt, Homo sapiens
  source 1..25: mol_type = other RNA
aacacccacctgctgtattatctcc

SEQ ID NO: 7 - RNA, 23 nt, Homo sapiens
  source 1..23: mol_type = other RNA
taaagtgaggacctgcactggta

SEQ ID NO: 8 - RNA, 25 nt, Homo sapiens
  source 1..25: mol_type = other RNA
atcctttggcccaccgtgttttctg

SEQ ID NO: 9 - RNA, 21 nt, Homo sapiens
  source 1..21: mol_type = other RNA
catcctttggcccaccgtgtt

SEQ ID NO: 10 - RNA, 25 nt, Homo sapiens
  source 1..25: mol_type = other RNA
gttacctctcttcatcctttggccc

SEQ ID NO: 11 - RNA, 25 nt, Homo sapiens
  source 1..25: mol_type = other RNA
ccaacatgcctaataatgaaaaagc

SEQ ID NO: 12 - RNA, 23 nt, Homo sapiens
  source 1..23: mol_type = other RNA
tttgtcagcagtcacattgccca

SEQ ID NO: 13 - RNA, 25 nt, Homo sapiens
  source 1..25: mol_type = other RNA
caatagacacatcggccacaccatc

SEQ ID NO: 14 - RNA, 23 nt, Homo sapiens
  source 1..23: mol_type = other RNA
tgatgcaatggtctcctgagagt

SEQ ID NO: 15 - RNA, 25 nt, Homo sapiens
  source 1..25: mol_type = other RNA
tccttttatgaaaacttaccaccag

SEQ ID NO: 16 - RNA, 25 nt, Homo sapiens
  source 1..25: mol_type = other RNA
tgatgatgccctgcactgggccgtc

SEQ ID NO: 17 - RNA, 25 nt, Homo sapiens
  source 1..25: mol_type = other RNA
cttgccttctgctcgaaattgatga

SEQ ID NO: 18 - RNA, 25 nt, Homo sapiens
  source 1..25: mol_type = other RNA
ccacctgctgtattatctccaaact

SEQ ID NO: 19 - RNA, 25 nt, Homo sapiens
  source 1..25: mol_type = other RNA
ttggcccaccgtgttttctggatag

SEQ ID NO: 20 - RNA, 25 nt, Homo sapiens
  source 1..25: mol_type = other RNA
attaggcatgttggagacttgggca

SEQ ID NO: 21 - RNA, 25 nt, Homo sapiens
  source 1..25: mol_type = other RNA
tgctgacaaagatggtgtggccgat

SEQ ID NO: 22 - DNA, 25 bp, Homo sapiens
  source 1..25: mol_type = other DNA
gtccattactttcctttaagaaaag

SEQ ID NO: 23 - DNA, 25 bp, Homo sapiens
  source 1..25: mol_type = other DNA
gtcctttaatgcttccccacacctt

SEQ ID NO: 24 - DNA, 22 bp, Homo sapiens
  source 1..22: mol_type = other DNA
caggcttcagtcagtcctttaa

SEQ ID NO: 25 - DNA, 26 bp, Homo sapiens
  source 1..26: mol_type = other DNA
actcatgaacatggaatccatgcagg

SEQ ID NO: 26 - DNA, 21 bp, Homo sapiens
  source 1..21: mol_type = other DNA
acacccacctgctgtattatc

SEQ ID NO: 27 - DNA, 25 bp, Homo sapiens
  source 1..25: mol_type = other DNA
aacacccacctgctgtattatctcc

SEQ ID NO: 28 - DNA, 23 bp, Homo sapiens
  source 1..23: mol_type = other DNA
taaagtgaggacctgcactggta

SEQ ID NO: 29 - DNA, 25 bp, Homo sapiens
  source 1..25: mol_type = other DNA
atcctttggcccaccgtgttttctg

SEQ ID NO: 30 - DNA, 21 bp, Homo sapiens
  source 1..21: mol_type = other DNA
catcctttggcccaccgtgtt

SEQ ID NO: 31 - DNA, 25 bp, Homo sapiens
  source 1..25: mol_type = other DNA
gttacctctcttcatcctttggccc

SEQ ID NO: 32 - DNA, 25 bp, Homo sapiens
  source 1..25: mol_type = other DNA
ccaacatgcctaataatgaaaaagc

SEQ ID NO: 33 - DNA, 23 bp, Homo sapiens
  source 1..23: mol_type = other DNA
tttgtcagcagtcacattgccca

SEQ ID NO: 34 - DNA, 25 bp, Homo sapiens
  source 1..25: mol_type = other DNA
caatagacacatcggccacaccatc

SEQ ID NO: 35 - DNA, 23 bp, Homo sapiens
  source 1..23: mol_type = other DNA
tgatgcaatggtctcctgagagt

SEQ ID NO: 36 - DNA, 25 bp, Homo sapiens
  source 1..25: mol_type = other DNA
tccttttatgaaaacttaccaccag

SEQ ID NO: 37 - DNA, 25 bp, Homo sapiens
  source 1..25: mol_type = other DNA
tgatgatgccctgcactgggccgtc

SEQ ID NO: 38 - DNA, 25 bp, Homo sapiens
  source 1..25: mol_type = other DNA
cttgccttctgctcgaaattgatga

SEQ ID NO: 39 - DNA, 25 bp, Homo sapiens
  source 1..25: mol_type = other DNA
ccacctgctgtattatctccaaact

SEQ ID NO: 40 - DNA, 25 bp, Homo sapiens
  source 1..25: mol_type = other DNA
ttggcccaccgtgttttctggatag

SEQ ID NO: 41 - DNA, 25 bp, Homo sapiens
  source 1..25: mol_type = other DNA
attaggcatgttggagacttgggca

SEQ ID NO: 42 - DNA, 25 bp, Homo sapiens
  source 1..25: mol_type = other DNA
tgctgacaaagatggtgtggccgat

SEQ ID NO: 43 - skipped

SEQ ID NO: 44 - RNA, 16 nt, Homo sapiens
  source 1..16: mol_type = other RNA
ctgctgtattatctcc

SEQ ID NO: 45 - DNA, 16 bp, Homo sapiens
  source 1..16: mol_type = other DNA
ctgctgtattatctcc

SEQ ID NO: 46 - DNA, 20 bp, Homo sapiens
  source 1..20: mol_type = other DNA
cgacgaaggccgtgtgcgtg

SEQ ID NO: 47 - DNA, 22 bp, Homo sapiens
  source 1..22: mol_type = other DNA
agttaaggggcctcagactaca